European Patent Application EP 4 414 458 A1, published August 14, 2024. Title: Collect & Extract - Lösung für die Sammlung und Lagerung biologischer Probentypen zur Extraktion von Biomolekülen. Applicant: Senckenberg Gesellschaft für Naturforschung. The sequence listing filed with the application follows.

SEQUENCE LISTING (8 sequences)

SEQ ID NO: 1 - DNA, 21 bp, synthetic construct
  source 1..21: mol_type = other DNA; note = L15995
ctccactatcagcacccaaag

SEQ ID NO: 2 - DNA, 20 bp, synthetic construct
  source 1..20: mol_type = other DNA; note = H16498
cctgaagtaagaaccagatg

SEQ ID NO: 3 - DNA, 17 bp, synthetic construct
  source 1..17: mol_type = other DNA; note = Chloroplast trnL Vorwaertsprimer
gggcaatcctgagccaa

SEQ ID NO: 4 - DNA, 22 bp, synthetic construct
  source 1..22: mol_type = other DNA; note = Chloroplast trnL Rueckwaertsprimer
ccattgagtctctgcacctatc

SEQ ID NO: 5 - DNA, 26 bp, synthetic construct
  source 1..26: mol_type = other DNA; note = Cytochrom Oxidase I Vorwaertsprimer
ggdacwggwtgaacwgtwtaycchcc

SEQ ID NO: 6 - DNA, 23 bp, synthetic construct
  source 1..23: mol_type = other DNA; note = Cytochrom Oxidase I Rueckwaertsprimer
gtratwgchccdgctarwacwgg

SEQ ID NO: 7 - DNA, 18 bp, synthetic construct
  source 1..18: mol_type = other DNA; note = ITS Vorwaertsprimer
gatgaagaacgyagyraa

SEQ ID NO: 8 - DNA, 20 bp, synthetic construct
  source 1..20: mol_type = other DNA; note = ITS Rueckwaertsprimer
tcctccgcttattgatatgc